European Patent Application EP 4 268 811 A1, published November 1, 2023. Title: A novel aminoalkanoic acid derivative containing a biphenyl group and an anti-inflammatory pharmaceutical composition comprising the same. Applicant: AmtixBio Co., Ltd. The sequence listing filed with the application follows.

SEQUENCE LISTING (14 sequences)

SEQ ID NO: 1 - DNA, 20 bp, Artificial Sequence
  Forward IL-17A
tctccaccgcaatgaagacc

SEQ ID NO: 2 - DNA, 20 bp, Artificial Sequence
  Reverse IL-17A
aaagtgaaggggcagctctc

SEQ ID NO: 3 - DNA, 21 bp, Artificial Sequence
  Forward IL-17F
tgctactgttgatgttgggac

SEQ ID NO: 4 - DNA, 21 bp, Artificial Sequence
  Reverse IL-17F
aatgccctggttttggttgaa

SEQ ID NO: 5 - DNA, 20 bp, Artificial Sequence
  Forward IL-23A p19
tggagcaacttcacacctcc

SEQ ID NO: 6 - DNA, 20 bp, Artificial Sequence
  Reverse IL-23A p19
ggcagctatggccaaaaagg

SEQ ID NO: 7 - DNA, 21 bp, Artificial Sequence
  Forward IL-12A p35
acctgctgaagaccacagatg

SEQ ID NO: 8 - DNA, 21 bp, Artificial Sequence
  Reverse IL-12A p35
gctccctcttgttgtggaaga

SEQ ID NO: 9 - DNA, 20 bp, Artificial Sequence
  Forward IL-12B p40
cctgtgacacgcctgaagaa

SEQ ID NO: 10 - DNA, 20 bp, Artificial Sequence
  Reverse IL-12B p40
gtgagtggctcagagtctcg

SEQ ID NO: 11 - DNA, 21 bp, Artificial Sequence
  Forward IL-1beta
ccaaaagatgaagggctgctt

SEQ ID NO: 12 - DNA, 23 bp, Artificial Sequence
  Reverse IL-1beta
gaaaagaaggtgctcatgtcctc

SEQ ID NO: 13 - DNA, 20 bp, Artificial Sequence
  Forward 18s rRNA
gtaacccgttgaaccccatt

SEQ ID NO: 14 - DNA, 20 bp, Artificial Sequence
  Reverse 18s rRNA
ccatccaatcggtagtagcg